European Patent Application EP 4 136 979 A1, published February 22, 2023. Title: Fermented milk. Applicant: GODO SHUSEI CO., Ltd. The sequence listing filed with the application follows.

SEQUENCE LISTING (2 sequences)

SEQ ID NO: 1 - DNA, 1379 bp, Trichoderma virens Gv29-8
atgctgtccaaggttgtctctctgctggctgccgccggcctggcctctgccgccgccgttgacaagagccactgcaagcctcccaagccttcctccaccatcactgtctgggagtctcagtacactgccaccggcactgctgctgttgctgctgctgctgccacggccaagaccagcagcccgaccagccacgtcaagggcaaggcctttgaccgctttgttgtcatttactttgagaaccaggactacgacaaggctgatggtgaccgtaagtttgaatctcgaatcctttgtctaaagaaggggacccggaagacgctgacagtatttgctttgcagccaacttcacttggttcgccaagaagggtgtcaagttgaccaactacttcggtgtcactcacccttctgagcccaactatatggccggtattattggtgactactttggcatgcagaacgatgacttcaactctgccgacttcaacgtgtccaccgtcatcgacctgctcgaggatcgtggcatctcttggggccactaccaggaggaccagccctacaccggctacgagggcttcagctacgtcaacaccaagaccggtgccaacgactacgtccgcaagcacaaccccgccatcttggccaacagcgtcacccactacgagcagcgcctgtcccaggtcaagaacctgtccatgatcgacaccggtcgctccatgttccacaaggacctcaaggacaacaagctgcctcagtggatgttcatcacccccaacatgacctctgacggccacgacaccaacgtcggcgttgctggcaagtggtgccgtgctttcctcgagcccctcctgaacgataagcacttcatggacaacacccttgtcctcctcacctgggatgagaacgagacctatgcccagcgcaaccagattctcgcaatcttgctcggtgacgccgtccccaagcaccttgttggcaccaccgacaacaacttctataaccactacagcgagatcgccaccgtcgaggccaactggaacctccacactctgggccgctgggatgttggtgccaacgtcttcgacctggttgccaaggagactggcgaccgcctccgcaagtggtcttccaccagggctgccaacagccacttctggaacgcctcttacgccggtgtcttcaacgaggagactggcaaccccaacaaccagtaccctgcccccaacctggctctcgaccgcagcttctctggccgtaccatcctgcccgccattaagaagacctgggagcacagcaagtctgccacctactacgccgacaccattgagctccccgacggcctgaaccctccccagggatacaagcccgtctccaccaactaa

SEQ ID NO: 2 - protein, 434 aa, Trichoderma virens Gv29-8
MLSKVVSLLAAAGLASAAAVDKSHCKPPKPSSTITVWESQYTATGTAAVAAAAATAKTSSPTSHVKGKAFDRFVVIYFENQDYDKADGDPNFTWFAKKGVKTNYFGVTHPSEPNYMAGIIGDYFGMQNDDFNSADFNVSTVIDLLEDRGISWGHYQEDQPYTGYEGFSYVNTKTGANDYVRKHNPAILANSVTHYEQRLSQVKNLSMIDTGRSMFHKDLKDNKLPQWMFITPNMTSDGHDTNVGVAGKWCRAFLEPLLNDKHFMDNTLVLLTWDENETYAQRNQILAILLGDAVPKHLVGTTDNNFYNHYSEIATVEANWNLHTLGRWDVGANVFDLVAKETGDRLRKWSSTRAANSHFWNASYAGVFNEETGNPNNQYPAPNLALDRSFSGRTILPAIKKTWEHSKSATYYADTIELPDGLNPPQGYKPVSTN